European Patent Application EP 4 248 738 A1, published September 27, 2023. Title: Cytoplasmic male sterile petunia plant, its intergeneric hybrid plant and method of producing the plant. Applicant: Sakata Seed Corporation. The sequence listing filed with the application follows.

SEQUENCE LISTING (82 sequences)

SEQ ID NO: 1 - DNA, 22 bp, Artificial Sequence
  primer
gctcaagcgcatcattttcgtg

SEQ ID NO: 2 - DNA, 22 bp, Artificial Sequence
  primer
catcaccggaaggatcgaaacc

SEQ ID NO: 3 - DNA, 21 bp, Artificial Sequence
  primer
aagctctaccaaggattgcca

SEQ ID NO: 4 - DNA, 20 bp, Artificial Sequence
  primer
gctgctttcgggtgattgga

SEQ ID NO: 5 - DNA, 20 bp, Artificial Sequence
  primer
cgccaactcctatcccgaag

SEQ ID NO: 6 - DNA, 19 bp, Artificial Sequence
  primer
cgtcgaagctaccgcgtat

SEQ ID NO: 7 - DNA, 20 bp, Artificial Sequence
  primer
ctggggttgaagaaggtccc

SEQ ID NO: 8 - DNA, 20 bp, Artificial Sequence
  primer
ttccagtcttcgaggcaagc

SEQ ID NO: 9 - DNA, 20 bp, Artificial Sequence
  primer
atcgggaattatgggctccg

SEQ ID NO: 10 - DNA, 21 bp, Artificial Sequence
  primer
agtaatgtgggttggcttgga

SEQ ID NO: 11 - DNA, 19 bp, Artificial Sequence
  primer
atggtgcggaaaaacccaa

SEQ ID NO: 12 - DNA, 25 bp, Artificial Sequence
  primer
atgatttctcgcaacagaattaagg

SEQ ID NO: 13 - DNA, 20 bp, Artificial Sequence
  primer
ctacaccgggggcaaaatct

SEQ ID NO: 14 - DNA, 20 bp, Artificial Sequence
  primer
gcgagcgcatccgattctaa

SEQ ID NO: 15 - DNA, 23 bp, Artificial Sequence
  primer
cgtctattaaggaggattccccg

SEQ ID NO: 16 - DNA, 20 bp, Artificial Sequence
  primer
gtcaggcccacctttcacaa

SEQ ID NO: 17 - DNA, 21 bp, Artificial Sequence
  primer
aggcaatccaatcttccgtgt

SEQ ID NO: 18 - DNA, 20 bp, Artificial Sequence
  primer
gaagcgattgcagcgaagaa

SEQ ID NO: 19 - DNA, 21 bp, Artificial Sequence
  primer
cttcggttagagcaaagccca

SEQ ID NO: 20 - DNA, 19 bp, Artificial Sequence
  primer
gcgtctgttcacggaggtt

SEQ ID NO: 21 - DNA, 20 bp, Artificial Sequence
  primer
tacaatgggagacgaaggcg

SEQ ID NO: 22 - DNA, 21 bp, Artificial Sequence
  primer
ttcgtacggagcaatcaacga

SEQ ID NO: 23 - DNA, 22 bp, Artificial Sequence
  primer
acagggaaggtggaagaaatga

SEQ ID NO: 24 - DNA, 20 bp, Artificial Sequence
  primer
aaatgccataaagcgcgacc

SEQ ID NO: 25 - DNA, 20 bp, Artificial Sequence
  primer
atagtgggggccgaatcaac

SEQ ID NO: 26 - DNA, 20 bp, Artificial Sequence
  primer
ttggagcagcaaactcggat

SEQ ID NO: 27 - DNA, 20 bp, Artificial Sequence
  primer
taagggggtgttcgagttgg

SEQ ID NO: 28 - DNA, 20 bp, Artificial Sequence
  primer
ccattcctcgtgagccactt

SEQ ID NO: 29 - DNA, 20 bp, Artificial Sequence
  primer
ggggtgcaacacttctcagt

SEQ ID NO: 30 - DNA, 21 bp, Artificial Sequence
  primer
ccagttacccggagttcaagt

SEQ ID NO: 31 - DNA, 20 bp, Artificial Sequence
  primer
gtaggtgatggggcatagcg

SEQ ID NO: 32 - DNA, 20 bp, Artificial Sequence
  primer
ccaactgagaccactcgacc

SEQ ID NO: 33 - DNA, 20 bp, Artificial Sequence
  primer
ccttggcctttggagaggag

SEQ ID NO: 34 - DNA, 21 bp, Artificial Sequence
  primer
ttccctctatcaggaacccgc

SEQ ID NO: 35 - DNA, 21 bp, Artificial Sequence
  primer
ctgctatcggtattggaaacg

SEQ ID NO: 36 - DNA, 20 bp, Artificial Sequence
  primer
atcgtggctttcaggttttg

SEQ ID NO: 37 - DNA, 21 bp, Artificial Sequence
  primer
ctttcgattcatttggctctc

SEQ ID NO: 38 - DNA, 21 bp, Artificial Sequence
  primer
ttccgttattgctgctggatt

SEQ ID NO: 39 - DNA, 20 bp, Artificial Sequence
  primer
tttcgcccttgctgctgtag

SEQ ID NO: 40 - DNA, 21 bp, Artificial Sequence
  primer
ttcacttccagttaggcagga

SEQ ID NO: 41 - DNA, 19 bp, Artificial Sequence
  primer
cccttgttagccgagctgt

SEQ ID NO: 42 - DNA, 20 bp, Artificial Sequence
  primer
aggcacggccatacataaga

SEQ ID NO: 43 - DNA, 20 bp, Artificial Sequence
  primer
agccgagaaggaagggatga

SEQ ID NO: 44 - DNA, 20 bp, Artificial Sequence
  primer
tcggtccaccctctagcttt

SEQ ID NO: 45 - DNA, 20 bp, Artificial Sequence
  primer
cgtcactggcctcccataag

SEQ ID NO: 46 - DNA, 20 bp, Artificial Sequence
  primer
tgcctctactccgcctactt

SEQ ID NO: 47 - DNA, 20 bp, Artificial Sequence
  primer
acacagcatacaggaggacg

SEQ ID NO: 48 - DNA, 20 bp, Artificial Sequence
  primer
tatgtggcagcgggaaagat

SEQ ID NO: 49 - DNA, 20 bp, Artificial Sequence
  primer
tcagccttccttatcgtggc

SEQ ID NO: 50 - DNA, 20 bp, Artificial Sequence
  primer
agtgcaggaaaggcagaagt

SEQ ID NO: 51 - DNA, 20 bp, Artificial Sequence
  primer
aggtcggccacaactcctat

SEQ ID NO: 52 - DNA, 21 bp, Artificial Sequence
  primer
tgctaaatctgagggtggcat

SEQ ID NO: 53 - DNA, 18 bp, Artificial Sequence
  primer
gcagaggtgacaaagcat

SEQ ID NO: 54 - DNA, 18 bp, Artificial Sequence
  primer
gaaaccaaacaaagagcg

SEQ ID NO: 55 - DNA, 20 bp, Artificial Sequence
  primer
gtggcgtatgtctacagcga

SEQ ID NO: 56 - DNA, 20 bp, Artificial Sequence
  primer
ggagccctgttcgagtgaaa

SEQ ID NO: 57 - DNA, 20 bp, Artificial Sequence
  primer
acctttgcttcgcccctatt

SEQ ID NO: 58 - DNA, 20 bp, Artificial Sequence
  primer
tagcactgctgccacttctg

SEQ ID NO: 59 - DNA, 20 bp, Artificial Sequence
  primer
acgtacctctcccgtaggtc

SEQ ID NO: 60 - DNA, 20 bp, Artificial Sequence
  primer
ctgtgaaacgaagcgcagag

SEQ ID NO: 61 - DNA, 20 bp, Artificial Sequence
  primer
ttcttactggatgcccggtg

SEQ ID NO: 62 - DNA, 19 bp, Artificial Sequence
  primer
tctcaccagcccgtagact

SEQ ID NO: 63 - DNA, 20 bp, Artificial Sequence
  primer
gcttcacagcgttgggctat

SEQ ID NO: 64 - DNA, 20 bp, Artificial Sequence
  primer
gagatccgcataagcaagcc

SEQ ID NO: 65 - DNA, 20 bp, Artificial Sequence
  primer
tgaggcagagtttcgtcctg

SEQ ID NO: 66 - DNA, 20 bp, Artificial Sequence
  primer
agcgcatagcggttttacga

SEQ ID NO: 67 - DNA, 20 bp, Artificial Sequence
  primer
gcattcccattgtaacggcg

SEQ ID NO: 68 - DNA, 20 bp, Artificial Sequence
  primer
tctactcgcctgcctacctt

SEQ ID NO: 69 - DNA, 19 bp, Artificial Sequence
  primer
gtcgatccaacgccgtctt

SEQ ID NO: 70 - DNA, 21 bp, Artificial Sequence
  primer
tccaatgcagtagcggtacac

SEQ ID NO: 71 - DNA, 22 bp, Artificial Sequence
  primer
ctaaggtggaagggaatggaga

SEQ ID NO: 72 - DNA, 20 bp, Artificial Sequence
  primer
gagcgaggtttgccattctt

SEQ ID NO: 73 - DNA, 20 bp, Artificial Sequence
  primer
gctagggaggaagccacttt

SEQ ID NO: 74 - DNA, 20 bp, Artificial Sequence
  primer
ctcagcttcgctcctcagtc

SEQ ID NO: 75 - DNA, 20 bp, Artificial Sequence
  primer
tcgctttcagttgaggtgga

SEQ ID NO: 76 - DNA, 20 bp, Artificial Sequence
  primer
tagattgagaggcgggaggt

SEQ ID NO: 77 - DNA, 20 bp, Artificial Sequence
  primer
gaagcagcggaacatgaagc

SEQ ID NO: 78 - DNA, 20 bp, Artificial Sequence
  primer
ataaagctgccctcccatcg

SEQ ID NO: 79 - DNA, 20 bp, Artificial Sequence
  primer
tgcggcgacaatacgttctt

SEQ ID NO: 80 - DNA, 20 bp, Artificial Sequence
  primer
atcgacggcattccaaaggt

SEQ ID NO: 81 - DNA, 20 bp, Artificial Sequence
  primer
tcataagcaaccgagcggaa

SEQ ID NO: 82 - DNA, 20 bp, Artificial Sequence
  primer
ccttcaccatgcctaccctg